European Patent Application EP 4 524 245 A1, published March 19, 2025. Title: IMMOBILIZED ENZYME, PREPARATION METHOD THEREFOR AND APPLICATION THEREOF. Applicant: ASYMCHEM LABORATORIES (TIANJIN) CO.,LTD. The sequence listing filed with the application follows.

SEQUENCE LISTING (8 sequences)

SEQ ID NO: 1 - protein, 338 aa, Sciscionella sp. SE31
MTTTEFANSNLVAVEPGAIREPTPPGSVIQYSEYELDRSQPLAGGVAWIEGEYVPADEARISIFDTGFGHSDLTYTVAHVWHGNIFRLEDHLDRLLHGAARLKLETGMSREELAGIAKRCVSLSQLREAYVNITITRGYGKKRGEKDLTKLTHQVYVYAIPYLWAFPPEEQIFGTSVIVPRHVRRAGRNTIDPTIKNYQWGDLTAASFEAKDRGARSAVLLDADNCVAEGPGFNVVLVKDGALVSPSRNALPGITRKTVYEIAAAKGIETMLRDVTSSELYEADELMAVTTAGGVTPITSLDGEQVGNGEPGPITVAIRDRFWALMDEPSSLIEAIDY

SEQ ID NO: 2 - protein, 253 aa, Acetobacter sp. CCTCC M209061
MTRVAGKVAIVSGAANGIGKATAQLLAKEGAKVVIGDLKEEDGQKAVAEIKAAGGEAAFVKLNVTDEAAWKAAIEQTLKLYGRLDIAVNNAGIAYSGSVESTSLEDWRRVQSINLDGVFLGTQVAIEAMKKSGGGSIVNLSSIEGLIGDPMGAAYNASKGGVRLFTKSAALHCAKSGYKIRVNSVHPGYIWTPMVAGLTKEDAAARQKLVDLHPIGHLGEPNDIAYGILYLASDESKFVTGSELVIDGGYTAQ

SEQ ID NO: 3 - protein, 603 aa, Rhodococcus ruber-SD1
MTTSIDREALRRKYAEERDKRIRPDGNDQYIRLDHVDGWSHDPYMPITPREPKLDHVTFAFIGGGFSGLVTAARLRESGVESVRIIDKAGDFGGVWYWNRYPGAMCDTAAMVYMPLLEETGYMPTEKYAHGPEILEHCQRIGKHYDLYDDALFHTEVTDLVWQEHDQRWRISTNRGDHFTAQFVGMGTGPLHVAQLPGIPGIESFRGKSFHTSRWDYDYTGGDALGAPMDKLADKRVAVIGTGATAVQCVPELAKYCRELYVVQRTPSAVDERGNHPIDEKWFAQIATPGWQKRWLDSFTAIWDGVLTDPSELAIEHEDLVQDGWTALGQRMRAAVGSVPIEQYSPENVQRALEEADDEQMERIRARVDEIVTDPATAAQLKAWFRQMCKRPCFHDDYLPAFNRPNTHLVDTGGKGVERITENGVVVAGVEYEVDCIVYASGFEFLGTGYTDRAGFDPTGRDGVKLSEHWAQGTRTLHGMHTYGFPNLFVLQLMQGAALGSNIPHNFVEAARVVAAIVDHVLSTGTSSVETTKEAEQAWVQLLLDHGRPLGNPECTPGYYNNEGKPAELKDRLNVGYPAGSAAFFRMMDHWLAAGSFDGLTFR

SEQ ID NO: 4 - protein, 353 aa, Chryseobacterium sp. CA49
MSTESLFTPFKYKNLELKNRIVMAPMTRAQSDNGVPTQQIADYYARRAAAEVGLILSEGTVINRPASKNMQNIPDFYGTEALNGWKNVIDAVHHNGGKMGPQIWHVGDTRSTPDYPLEDMEKASTMTLEDIQDTIAQFAASAKSAKDLGFDVLEIHGAHGYLIDQFFWEGTNTRTDEYGGKTIKERSRFAVDVVKAIRAAVGEDFTIIIRLSQWKQQDYSVKLAHTPEEMEEWLLPLKDAGVDIFHCSQRRFWEPEFEGSDLNFAGWAKKITGQPTITVGSVGLEGDFMAAFGGQGTEKADLTELTKRLERGDFDLVAVGRALLQDPEWAKKVKEQNTEALLDFSAESLGVLY

SEQ ID NO: 5 - protein, 285 aa, Amycolatopsis decaplanina
MSPGGTLTLGDLTVSRMGYGAMRLSGPGIWGPPSDRETAIAVLREAVELGVTHIDTSDFYGPHTVNELIREALHPYPDELHIVTKVGAKRSPDKGWPSALSREELTSAVHDNLRNLGVDVLDVVNLRLAGEHGVFPIPVSITEPFEVLAELRQQGLIRHLGLSHVSAEQVKEARAIAPVVCVQNEYNVANRANDDLLDALAAINIPFVPYFPLGGFTPLQSGVLDDCARRVDATPMQVALAWLLQRSPNILVIPGTSSPSHLRENVAAAKLELPADVIADLDALV

SEQ ID NO: 6 - protein, 299 aa, Saccharothrix syringae
MTDNALAQPGPSTPLTLLGTGAMGTALARAWLAAGHPVTVWNRTPARAEALAAEGATVAASAAEAVAANRLVVVCLLDDASVGEALDGADLTGRDLVNITTGTPGQGRSRAAWAKARGARFLDGGIMAVPPMIGAPDSGAYVFYSGSAALFEEHRDTLAVPAGTTYVGADPGFAALHDVALLSAMNGMFAGITHAFALIRREDIAPKDFAPLLVSWLTAMAHSAHKAADQLESGDYGKDVVSSLAMQVAGNATLLRTAEEQGVSAELLRPYMDLMERRLALGNGEEDTTGVVELLLRKP

SEQ ID NO: 7 - protein, 366 aa, Thermoactinomyces intermedius ATCC33205
MRDVFEMMDRYGHEQVIFCRHPQTGLKAIIALHNTTAGPALGGCRMIPYASTDEALEDVLRLSKGMTYKCSLADVDFGGGKMVIIGDPKKDKSPELFRVIGRFVGGLNGRFYTGTDMGTNPEDFVHAARESKSFAGLPKSYGGKGDTSIPTALGVFHGMRATARFLWGTDQLKGRVVAIQGVGKVGERLLQLLVEVGAYCKIADIDSVRCEQLKEKYGDKVQLVDVNRIHKESCDIFSPCAKGGVVNDDTIDEFRCLAIVGSANNQLVEDRHGALLQKRSICYAPDYLVNAGGLIQVADELEGFHEERVLAKTEAIYDMVLDIFHRAKNENITTCEAADRIVMERLKKLTDIRRILLEDPRNSARR

SEQ ID NO: 8 - protein, 318 aa, 2 Ambystoma laterale x Ambystoma jeffersonianum
MLPSGSDPAFSQPKSVLDAGLTCQGASPSSVSKPILLVPGTGTTGPQSFDSNWIPLSTQLGYTPCWISPPPFMLNDTQVNTEYMVNAITALYAGSGNNKLPVLTWSQGGLVAQWGLTFFPSIRSKVDRLMAFAPDYKGTVLAGPLDALAVSAPSVWQQTTGSALTTALRNAGGLTQIVPTTNLYSATDEIVQPQVSNSPLDSSYLFNGKNVQAQAVCGPLFVIDHAGSLTSQFSYVVGRSALRSTTGQARSADYGITDCNPLPANDLTPEQKVAAAALLAPAAAAIVAGPKQNCEPDLMPYARPFAVGKRTCSGIVTP